European Patent Application EP 4 483 959 A2, published January 1, 2025. Title: NOVEL PEPTIDE COMPOUND OR PHARMACEUTICALLY ACCEPTABLE SALT THEREOF. Applicant: EYEBIO KOREA. Application EP. The sequence listing filed with the application follows.

SEQUENCE LISTING (116 sequences)

SEQ ID NO: 1 - protein, 5 aa, synthetic construct
  REGION 1..5: note = Example 10
  SITE 1: note = MISC_FEATURE - P at position 1 is (2S,4R) trans-4-hydroxy-L-proline.
PGQDG

SEQ ID NO: 2 - protein, 6 aa, synthetic construct
  REGION 1..6: note = Example 11
  SITE 1: note = MISC_FEATURE - P at position 1 is (2S,4R) trans-4-hydroxy-L-proline.
PGQDGL

SEQ ID NO: 3 - protein, 7 aa, synthetic construct
  REGION 1..7: note = Example 12
  SITE 1: note = MISC_FEATURE - P at position 1 is (2S,4R) trans-4-hydroxy-L-proline.
PGQDGLA

SEQ ID NO: 4 - protein, 5 aa, synthetic construct
  REGION 1..5: note = Example 13
  SITE 1: note = MISC_FEATURE - P at position 1 is (2S,4R) trans-4-hydroxy-L-proline.
PGQAG

SEQ ID NO: 5 - protein, 7 aa, synthetic construct
  REGION 1..7: note = Example 14
  SITE 1: note = MISC_FEATURE - P at position 1 is (2S,4R) trans-4-hydroxy-L-proline.
PGQAGLA

SEQ ID NO: 6 - protein, 8 aa, synthetic construct
  REGION 1..8: note = Example 15
  SITE 1: note = MISC_FEATURE - P at position 1 is (2S,4R) trans-4-hydroxy-L-proline.
PGQDGLAG

SEQ ID NO: 7 - protein, 8 aa, synthetic construct
  REGION 1..8: note = Example 16
QDGLAGPK

SEQ ID NO: 8 - protein, 8 aa, synthetic construct
  REGION 1..8: note = Example 17
  SITE 1: note = MISC_FEATURE - P at position 1 is (2S,4R) trans-4-hydroxy-L-proline.
PGQLGLAG

SEQ ID NO: 9 - protein, 8 aa, synthetic construct
  REGION 1..8: note = Example 18
QLGLAGPK

SEQ ID NO: 10 - protein, 7 aa, synthetic construct
  REGION 1..7: note = Example 19
DGLAGPK

SEQ ID NO: 11 - protein, 7 aa, synthetic construct
  REGION 1..7: note = Example 20
LGLAGPK

SEQ ID NO: 12 - protein, 5 aa, synthetic construct
  REGION 1..5: note = Example 21
  SITE 1: note = MISC_FEATURE - P at position 1 is (2S,4R) trans-4-hydroxy-L-proline.
PGQDV

SEQ ID NO: 13 - protein, 6 aa, synthetic construct
  SITE 1: note = MISC_FEATURE - P at position 1 is (2S,4R) trans-4-hydroxy-L-proline.
PGQDVL

SEQ ID NO: 14 - protein, 7 aa, synthetic construct
  REGION 1..7: note = Example 23
  SITE 1: note = MISC_FEATURE - P at position 1 is (2S,4R) trans-4-hydroxy-L-proline.
PGQDVLA

SEQ ID NO: 15 - protein, 8 aa, synthetic construct
  REGION 1..8: note = Example 24
  SITE 1: note = MISC_FEATURE - P at position 1 is (2S,4R) trans-4-hydroxy-L-proline.
PGQDVLAG

SEQ ID NO: 16 - protein, 5 aa, synthetic construct
  REGION 1..5: note = Example 25
LAGPK

SEQ ID NO: 17 - protein, 6 aa, synthetic construct
  REGION 1..6: note = Example 26
GLAGPK

SEQ ID NO: 18 - protein, 7 aa, synthetic construct
  REGION 1..7: note = Example 27
  SITE 1: note = MISC_FEATURE - P at position 1 is (2S,4R) trans-4-hydroxy-L-proline.
PGLAGPK

SEQ ID NO: 19 - protein, 7 aa, synthetic construct
  REGION 1..7: note = Example 28
  SITE 1: note = MISC_FEATURE - P at position 1 is (2S,4R) trans-4-hydroxy-L-proline.
PGQDGPK

SEQ ID NO: 20 - protein, 6 aa, synthetic construct
  REGION 1..6: note = Example 29
GQDGLA

SEQ ID NO: 21 - protein, 6 aa, synthetic construct
  REGION 1..6: note = Example 30
QDGLAG

SEQ ID NO: 22 - protein, 6 aa, synthetic construct
  REGION 1..6: note = Example 31
DGLAGP

SEQ ID NO: 23 - protein, 5 aa, synthetic construct
  REGION 1..5: note = Example 32
  SITE 1: note = MISC_FEATURE - P at position 1 is (2S,4R) trans-4-hydroxy-L-proline.
PGQDL

SEQ ID NO: 24 - protein, 5 aa, synthetic construct
  REGION 1..5: note = Example 33
  SITE 1: note = MISC_FEATURE - P at position 1 is (2S,4R) trans-4-hydroxy-L-proline.
PGQDA

SEQ ID NO: 25 - protein, 6 aa, synthetic construct
  REGION 1..6: note = Example 34
  SITE 1: note = MISC_FEATURE - P at position 1 is (2S,4R) trans-4-hydroxy-L-proline.
PGQDVL

SEQ ID NO: 26 - protein, 6 aa, synthetic construct
  REGION 1..6: note = Example 35
  SITE 1: note = MISC_FEATURE - P at position 1 is (2S,4R) trans-4-hydroxy-L-proline.
PGQDLL

SEQ ID NO: 27 - protein, 6 aa, synthetic construct
  REGION 1..6: note = Example 36
  SITE 1: note = MISC_FEATURE - P at position 1 is (2S,4R) trans-4-hydroxy-L-proline.
PGQDAL

SEQ ID NO: 28 - protein, 7 aa, synthetic construct
  REGION 1..7: note = Example 37
  SITE 1: note = MISC_FEATURE - P at position 1 is (2S,4R) trans-4-hydroxy-L-proline.
PGQDVLA

SEQ ID NO: 29 - protein, 7 aa, synthetic construct
  REGION 1..7: note = Example 38
  SITE 1: note = MISC_FEATURE - P at position 1 is (2S,4R) trans-4-hydroxy-L-proline.
PGQDLLA

SEQ ID NO: 30 - protein, 7 aa, synthetic construct
  REGION 1..7: note = Example 39
  SITE 1: note = MISC_FEATURE - P at position 1 is (2S,4R) trans-4-hydroxy-L-proline.
PGQDALA

SEQ ID NO: 31 - protein, 5 aa, synthetic construct
  REGION 1..5: note = Example 40
  SITE 1: note = MISC_FEATURE - P at position 1 is trans-4-Hydroxy-D-proline.
PGQDG

SEQ ID NO: 32 - protein, 5 aa, synthetic construct
  REGION 1..5: note = Example 41
  SITE 1: note = MISC_FEATURE - P at position 1 is cis-4-fluoro-L-proline.
PGQDG

SEQ ID NO: 33 - protein, 5 aa, synthetic construct
  REGION 1..5: note = Example 42
  SITE 1: note = MISC_FEATURE - P at position 1 is trans-4-amino-L-proline.
PGQDG

SEQ ID NO: 34 - protein, 5 aa, synthetic construct
  REGION 1..5: note = Example 43
  SITE 1: note = MISC_FEATURE - P at position 1 is 4-difluoro-L-proline.
PGQDG

SEQ ID NO: 35 - protein, 5 aa, synthetic construct
  REGION 1..5: note = Example 44
  SITE 1: note = MISC_FEATURE - P at position 1 is 4-methylene-L-proline.
PGQDG

SEQ ID NO: 36 - protein, 6 aa, synthetic construct
  REGION 1..6: note = Example 45
  SITE 1: note = MISC_FEATURE - P at position 1 is trans-4-Hydroxy-D-proline.
PGQDGL

SEQ ID NO: 37 - protein, 6 aa, synthetic construct
  REGION 1..6: note = Example 46
  SITE 1: note = MISC_FEATURE - P at position 1 is cis-4-fluoro-L-proline.
PGQDGL

SEQ ID NO: 38 - protein, 6 aa, synthetic construct
  REGION 1..6: note = Example 47
  SITE 1: note = MISC_FEATURE - P at position 1 is trans-4-amino-L-proline.
PGQDGL

SEQ ID NO: 39 - protein, 6 aa, synthetic construct
  REGION 1..6: note = Example 48
  SITE 1: note = MISC_FEATURE - P at position 1 is 4-difluoro-L-proline.
PGQDGL

SEQ ID NO: 40 - protein, 6 aa, synthetic construct
  REGION 1..6: note = Example 49
  SITE 1: note = MISC_FEATURE - P at position 1 is 4-methylene-L-proline.
PGQDGL

SEQ ID NO: 41 - protein, 7 aa, synthetic construct
  REGION 1..7: note = Example 50
  SITE 1: note = MISC_FEATURE - P at position 1 is trans-4-hydroxy-D-proline.
PGQDGLA

SEQ ID NO: 42 - protein, 7 aa, synthetic construct
  REGION 1..7: note = Example 51
  SITE 1: note = MISC_FEATURE - P at position 1 is cis-4-fluoro-L-proline.
PGQDGLA

SEQ ID NO: 43 - protein, 7 aa, synthetic construct
  REGION 1..7: note = Example 52
  SITE 1: note = MISC_FEATURE - P at position 1 is trans-4-amino-L-proline.
PGQDGLA

SEQ ID NO: 44 - protein, 7 aa, synthetic construct
  REGION 1..7: note = Example 53
  SITE 1: note = MISC_FEATURE - P at position 1 is 4-difluoro-L-proline.
PGQDGLA

SEQ ID NO: 45 - protein, 7 aa, synthetic construct
  REGION 1..7: note = Example 54
  SITE 1: note = MISC_FEATURE - P at position 1 is 4-methylene-L-proline.
PGQDGLA

SEQ ID NO: 46 - protein, 5 aa, synthetic construct
  REGION 1..5: note = Example 55
  SITE 1: note = MISC_FEATURE - P at position 1 is 4,4-dimethyl-L-proline.
PGQDG

SEQ ID NO: 47 - protein, 6 aa, synthetic construct
  REGION 1..6: note = Example 56
  SITE 1: note = MISC_FEATURE - P at position 1 is 4,4-dimethyl-L-proline.
PGQDGL

SEQ ID NO: 48 - protein, 7 aa, synthetic construct
  REGION 1..7: note = Example 57
  SITE 1: note = MISC_FEATURE - P at position 1 is 4,4-dimethyl-L-proline.
PGQDGLA

SEQ ID NO: 49 - protein, 5 aa, synthetic construct
  REGION 1..5: note = Example 58
  SITE 1: note = MISC_FEATURE - P at position 1 is (2S,4R) trans-4-hydroxy-L-proline.
  SITE 3: note = MISC_FEATURE - Q at position 3 is D-glutamine.
PGQDG

SEQ ID NO: 50 - protein, 5 aa, synthetic construct
  REGION 1..5: note = Example 59
  SITE 1: note = MISC_FEATURE - P at position 1 is (2S,4R) trans-4-hydroxy-L-proline.
  SITE 4: note = MISC_FEATURE - D at position 4 is D-aspartic acid.
PGQDG

SEQ ID NO: 51 - protein, 6 aa, synthetic construct
  REGION 1..6: note = Example 60
  SITE 1: note = MISC_FEATURE - P at position 1 is (2S,4R) trans-4-hydroxy-L-proline.
  SITE 3: note = MISC_FEATURE - Q at position 3 is D-glutamine.
PGQDGL

SEQ ID NO: 52 - protein, 6 aa, synthetic construct
  REGION 1..6: note = Example 61
  SITE 1: note = MISC_FEATURE - P at position 1 is (2S,4R) trans-4-hydroxy-L-proline.
  SITE 4: note = MISC_FEATURE - D at position 4 is D-aspartic acid.
PGQDGL

SEQ ID NO: 53 - protein, 6 aa, synthetic construct
  REGION 1..6: note = Example 62
  SITE 1: note = MISC_FEATURE - P at position 1 is (2S,4R) trans-4-hydroxy-L-proline.
  SITE 6: note = MISC_FEATURE - L at position 6 is D-leucine.
PGQDGL

SEQ ID NO: 54 - protein, 7 aa, synthetic construct
  REGION 1..7: note = Example 63
  SITE 1: note = MISC_FEATURE - P at position 1 is (2S,4R) trans-4-hydroxy-L-proline.
  SITE 3: note = MISC_FEATURE - Q at position 3 is D-glutamine.
PGQDGLA

SEQ ID NO: 55 - protein, 7 aa, synthetic construct
  REGION 1..7: note = Example 64
  SITE 1: note = MISC_FEATURE - P at position 1 is (2S,4R) trans-4-hydroxy-L-proline.
  SITE 4: note = MISC_FEATURE - D at position 4 is D-aspartic acid.
PGQDGLA

SEQ ID NO: 56 - protein, 7 aa, synthetic construct
  REGION 1..7: note = Example 65
  SITE 1: note = MISC_FEATURE - P at position 1 is (2S,4R) trans-4-hydroxy-L-proline.
  SITE 6: note = MISC_FEATURE - L at position 6 is D-leucine.
PGQDGLA

SEQ ID NO: 57 - protein, 7 aa, synthetic construct
  REGION 1..7: note = Example 66
  SITE 1: note = MISC_FEATURE - P at position 1 is (2S,4R) trans-4-hydroxy-L-proline.
  SITE 7: note = MISC_FEATURE - A at position 7 is D-alanine.
PGQDGLA

SEQ ID NO: 58 - protein, 5 aa, synthetic construct
  REGION 1..5: note = Example 67
  SITE 1: note = MISC_FEATURE - P at position 1 is (2S,4R) trans-4-hydroxy-L-proline.
PGQEG

SEQ ID NO: 59 - protein, 6 aa, synthetic construct
  REGION 1..6: note = Example 68
  SITE 1: note = MISC_FEATURE - P at position 1 is (2S,4R) trans-4-hydroxy-L-proline.
PGQEGL

SEQ ID NO: 60 - protein, 7 aa, synthetic construct
  REGION 1..7: note = Example 69
  SITE 1: note = MISC_FEATURE - P at position 1 is (2S,4R) trans-4-hydroxy-L-proline.
PGQEGLA

SEQ ID NO: 61 - protein, 6 aa, synthetic construct
  REGION 1..6: note = Example 70
QEGLAG

SEQ ID NO: 62 - protein, 6 aa, synthetic construct
  REGION 1..6: note = Example 71
  SITE 1: note = MISC_FEATURE - P at position 1 is (2S,4R) trans-4-hydroxy-L-proline.
PGQDGV

SEQ ID NO: 63 - protein, 7 aa, synthetic construct
  REGION 1..7: note = Example 72
  SITE 1: note = MISC_FEATURE - P at position 1 is (2S,4R) trans-4-hydroxy-L-proline.
PGQDGVA

SEQ ID NO: 64 - protein, 5 aa, synthetic construct
  REGION 1..5: note = Example 73
  SITE 1: note = MISC_FEATURE - P at position 1 is (2S,4R) trans-4-hydroxy-L-proline.
PAQDG

SEQ ID NO: 65 - protein, 5 aa, synthetic construct
  REGION 1..5: note = Example 74
  SITE 1: note = MISC_FEATURE - P at position 1 is (2S,4R) trans-4-hydroxy-L-proline.
PVQDG

SEQ ID NO: 66 - protein, 5 aa, synthetic construct
  REGION 1..5: note = Example 75
  SITE 1: note = MISC_FEATURE - P at position 1 is (2S,4R) trans-4-hydroxy-L-proline.
PLQDG

SEQ ID NO: 67 - protein, 5 aa, synthetic construct
  REGION 1..5: note = Example 76
PGQDG

SEQ ID NO: 68 - protein, 6 aa, synthetic construct
  REGION 1..6: note = Example 77
PGQDGL

SEQ ID NO: 69 - protein, 7 aa, synthetic construct
  REGION 1..7: note = Example 78
PGQDGLA

SEQ ID NO: 70 - protein, 7 aa, synthetic construct
  REGION 1..7: note = Example 79
  SITE 1: note = MISC_FEATURE - P at position 1 is (2S,4R) trans-4-hydroxy-L-proline.
PGQNGLA

SEQ ID NO: 71 - protein, 7 aa, synthetic construct
  REGION 1..7: note = Example 80
  SITE 1: note = MISC_FEATURE - P at position 1 is (2S,4R) trans-4-hydroxy-L-proline.
PGQHGLA

SEQ ID NO: 72 - protein, 6 aa, synthetic construct
  REGION 1..6: note = Example 81
  SITE 1: note = MISC_FEATURE - P at position 1 is (2S,4R) trans-4-hydroxy-L-proline.
PGQNGL

SEQ ID NO: 73 - protein, 6 aa, synthetic construct
  REGION 1..6: note = Example 82
  SITE 1: note = MISC_FEATURE - P at position 1 is (2S,4R) trans-4-hydroxy-L-proline.
PGQHGL

SEQ ID NO: 74 - protein, 7 aa, synthetic construct
  REGION 1..7: note = Example 83
  SITE 1: note = MISC_FEATURE - P at position 1 is (2S,4R) trans-4-hydroxy-L-proline.
  SITE 5: note = MISC_FEATURE - Xaa at position 5 is 2-aminoisobutyric acid.
PGQDXLA

SEQ ID NO: 75 - protein, 6 aa, synthetic construct
  REGION 1..6: note = Example 84
  SITE 1: note = MISC_FEATURE - P at position 1 is (2S,4R) trans-4-hydroxy-L-proline.
  SITE 4: note = MISC_FEATURE - Xaa at position 4 is 2-aminoisobutyric acid.
PGQXGL

SEQ ID NO: 76 - protein, 5 aa, synthetic construct
  REGION 1..5: note = Example 85
  SITE 1: note = MISC_FEATURE - P at position 1 is (2S,4R) trans-4-hydroxy-L-proline.
  SITE 5: note = MISC_FEATURE - Xaa at position 5 is 2-aminoisobutyric acid.
PGQDX

SEQ ID NO: 77 - protein, 7 aa, synthetic construct
  REGION 1..7: note = Example 86
  SITE 1: note = MISC_FEATURE - P at position 1 is (2S,4R) trans-4-hydroxy-L-proline.
PGQELLA

SEQ ID NO: 78 - protein, 7 aa, synthetic construct
  REGION 1..7: note = Example 87
  SITE 1: note = MISC_FEATURE - P at position 1 is (2S,4R) trans-4-hydroxy-L-proline.
PGQEVLA

SEQ ID NO: 79 - protein, 6 aa, synthetic construct
  REGION 1..6: note = Example 88
  SITE 1: note = MISC_FEATURE - P at position 1 is (2S,4R) trans-4-hydroxy-L-proline.
PGQELL

SEQ ID NO: 80 - protein, 6 aa, synthetic construct
  REGION 1..6: note = Example 89
  SITE 1: note = MISC_FEATURE - P at position 1 is (2S,4R) trans-4-hydroxy-L-proline.
PGQEVL

SEQ ID NO: 81 - protein, 5 aa, synthetic construct
  REGION 1..5: note = Example 90
  SITE 1: note = MISC_FEATURE - P at position 1 is (2S,4R) trans-4-hydroxy-L-proline.
PGQEL

SEQ ID NO: 82 - protein, 5 aa, synthetic construct
  REGION 1..5: note = Example 91
  SITE 1: note = MISC_FEATURE - P at position 1 is (2S,4R) trans-4-hydroxy-L-proline.
PGQEV

SEQ ID NO: 83 - protein, 7 aa, synthetic construct
  REGION 1..7: note = Example 92
  SITE 1: note = MISC_FEATURE - P at position 1 is (2S,4R) trans-4-hydroxy-L-proline.
  SITE 5: note = MISC_FEATURE - Xaa at position 5 is 2-aminoisobutyric acid.
PGQEXLA

SEQ ID NO: 84 - protein, 7 aa, synthetic construct
  REGION 1..7: note = Example 93
  SITE 1: note = MISC_FEATURE - P at position 1 is (2S,4R) trans-4-hydroxy-L-proline.
  SITE 5: note = MISC_FEATURE - Xaa at position 5 is L-a-tert-butylglycine.
PGQEXLA

SEQ ID NO: 85 - protein, 7 aa, synthetic construct
  REGION 1..7: note = Example 94
  SITE 1: note = MISC_FEATURE - P at position 1 is (2S,4R) trans-4-hydroxy-L-proline
  SITE 5: note = MISC_FEATURE - Xaa at position 5 is phenylglycine.
PGQEXLA

SEQ ID NO: 86 - protein, 5 aa, synthetic construct
  REGION 1..5: note = Example 95
  SITE 1: note = MISC_FEATURE - P at position 1 is (2S,4R) trans-4-hydroxy-L-proline.
PGQLV

SEQ ID NO: 87 - protein, 7 aa, synthetic construct
  REGION 1..7: note = Example 96
  SITE 1: note = MISC_FEATURE - P at position 1 is (2S,4R) trans-4-hydroxy-L-proline.
PGQLLLA

SEQ ID NO: 88 - protein, 7 aa, synthetic construct
  REGION 1..7: note = Example 97
  SITE 1: note = MISC_FEATURE - P at position 1 is (2S,4R) trans-4-hydroxy-L-proline.
PGQLVLA

SEQ ID NO: 89 - protein, 6 aa, synthetic construct
  REGION 1..6: note = Example 98
  SITE 1: note = MISC_FEATURE - P at position 1 is (2S,4R) trans-4-hydroxy-L-proline.
PGQLLL

SEQ ID NO: 90 - protein, 6 aa, synthetic construct
  REGION 1..6: note = Example 99
  SITE 1: note = MISC_FEATURE - P at position 1 is (2S,4R) trans-4-hydroxy-L-proline.
PGQLVL

SEQ ID NO: 91 - protein, 5 aa, synthetic construct
  REGION 1..5: note = Example 100
  SITE 1: note = MISC_FEATURE - P at position 1 is (2S,4R) trans-4-hydroxy-L-proline.
  SITE 4: note = MISC_FEATURE - Xaa at position 4 is apartimide or aminosuccinimide.
PGQXG

SEQ ID NO: 92 - protein, 6 aa, synthetic construct
  REGION 1..6: note = Example 101
  SITE 1: note = MISC_FEATURE - P at position 1 is (2S,4R) trans-4-hydroxy-L-proline.
  SITE 4: note = MISC_FEATURE - Xaa at position 4 is apartimide or aminosuccinimide.
PGQXGL

SEQ ID NO: 93 - protein, 7 aa, synthetic construct
  REGION 1..7: note = Example 102
  SITE 1: note = MISC_FEATURE - P at position 1 is (2S,4R) trans-4-hydroxy-L-proline.
  SITE 4: note = MISC_FEATURE - Xaa at position 4 is apartimide or aminosuccinimide.
PGQXGLA

SEQ ID NO: 94 - protein, 8 aa, synthetic construct
  REGION 1..8: note = Example 103
  SITE 1: note = MISC_FEATURE - P at position 1 is (2S,4R) trans-4-hydroxy-L-proline.
  SITE 4: note = MISC_FEATURE - Xaa at position 4 is apartimide or aminosuccinimide
PGQXGLAG

SEQ ID NO: 95 - protein, 8 aa, synthetic construct
  REGION 1..8: note = Example 104
  SITE 2: note = MISC_FEATURE - Xaa at position 2 is apartimide or aminosuccinimide.
QXGLAGPK

SEQ ID NO: 96 - protein, 7 aa, synthetic construct
  REGION 1..7: note = Example 105
  SITE 1: note = MISC_FEATURE - Xaa at position 1 is apartimide or aminosuccinimide.
XGLAGPK

SEQ ID NO: 97 - protein, 5 aa, synthetic construct
  REGION 1..5: note = Example 106
  SITE 1: note = MISC_FEATURE - P at position 1 is (2S,4R) trans-4-hydroxy-L-proline.
  SITE 5: note = MISC_FEATURE - G at position 5 is glycine substituted with isopropyl ester.
PGQDG

SEQ ID NO: 98 - protein, 6 aa, synthetic construct
  REGION 1..6: note = Example 107
  SITE 1: note = MISC_FEATURE - P at position 1 is (2S,4R) trans-4-hydroxy-L-proline.
  SITE 6: note = MISC_FEATURE - L at position 6 is leucine substituted with isopropyl ester.
PGQDGL

SEQ ID NO: 99 - protein, 7 aa, synthetic construct
  REGION 1..7: note = Example 108
  SITE 1: note = MISC_FEATURE - P at position 1 is (2S,4R) trans-4-hydroxy-L-proline.
  SITE 7: note = MISC_FEATURE - A at position 7 is alanine substituted with isopropyl ester.
PGQDGLA

SEQ ID NO: 100 - protein, 5 aa, synthetic construct
  REGION 1..5: note = Example 109
  SITE 1: note = MISC_FEATURE - P at position 1 is (2S,4R) trans-4-hydroxy-L-proline.
  SITE 4: note = MISC_FEATURE - Xaa at position 4 is apartimide or aminosuccinimide.
  SITE 5: note = MISC_FEATURE - G at position 5 is glycine substituted with isopropyl ester.
PGQXG

SEQ ID NO: 101 - protein, 5 aa, synthetic construct
  REGION 1..5: note = Example 110
  SITE 1: note = MISC_FEATURE - P at position 1 is (2S,4R) trans-4-hydroxy-L-proline.
  SITE 4: note = MISC_FEATURE - D at position 4 is aspartic acid substituted with isopropyl ester.
  SITE 5: note = MISC_FEATURE - G at position 5 is glycine substituted with isopropyl ester.
PGQDG

SEQ ID NO: 102 - protein, 6 aa, synthetic construct
  REGION 1..6: note = Example 111
  SITE 1: note = MISC_FEATURE - P at position 1 is (2S,4R) trans-4-hydroxy-L-proline.
  SITE 4: note = MISC_FEATURE - Xaa at position 4 is apartimide or aminosuccinimide.
  SITE 6: note = MISC_FEATURE - L at position 6 is leucine substituted with isopropyl ester.
PGQXGL

SEQ ID NO: 103 - protein, 6 aa, synthetic construct
  REGION 1..6: note = Example 112
  SITE 1: note = MISC_FEATURE - P at position 1 is (2S,4R) trans-4-hydroxy-L-proline.
  SITE 4: note = MISC_FEATURE - D at position 4 is aspartic acid substituted with isopropyl ester.
  SITE 6: note = MISC_FEATURE - L at position 6 is leucine substituted with isopropyl ester.
PGQDGL

SEQ ID NO: 104 - protein, 7 aa, synthetic construct
  REGION 1..7: note = Example 113
  SITE 1: note = MISC_FEATURE - P at position 1 is (2S,4R) trans-4-hydroxy-L-proline.
  SITE 4: note = MISC_FEATURE - Xaa at position 4 is apartimide or aminosuccinimide.
  SITE 7: note = MISC_FEATURE - A at position 7 is alanine substituted with isopropyl ester.
PGQXGLA

SEQ ID NO: 105 - protein, 7 aa, synthetic construct
  REGION 1..7: note = Example 114
  SITE 1: note = MISC_FEATURE - P at position 1 is (2S,4R) trans-4-hydroxy-L-proline.
  SITE 4: note = MISC_FEATURE - D at position 4 is aspartic acid substituted with isopropyl ester.
  SITE 7: note = MISC_FEATURE - A at position 7 is alanine substituted with isopropyl ester.
PGQDGLA

SEQ ID NO: 106 - protein, 5 aa, synthetic construct
  REGION 1..5: note = Example 115
  SITE 1: note = MISC_FEATURE - P at position 1 is (2S,4R) trans-4-hydroxy-L-proline.
  SITE 4: note = MISC_FEATURE - D at position 4 is aspartic acid substituted with isopropyl ester.
PGQDG

SEQ ID NO: 107 - protein, 6 aa, synthetic construct
  REGION 1..6: note = Example 116
  SITE 1: note = MISC_FEATURE - P at position 1 is (2S,4R) trans-4-hydroxy-L-proline.
  SITE 4: note = MISC_FEATURE - D at position 4 is aspartic acid substituted with isopropyl ester.
PGQDGL

SEQ ID NO: 108 - protein, 7 aa, synthetic construct
  REGION 1..7: note = Example 117
  SITE 1: note = MISC_FEATURE - P at position 1 is (2S,4R) trans-4-hydroxy-L-proline.
  SITE 4: note = MISC_FEATURE - D at position 4 is aspartic acid substituted with isopropyl ester.
PGQDGLA

SEQ ID NO: 109 - protein, 6 aa, synthetic construct
  REGION 1..6: note = Example 118
  SITE 2: note = MISC_FEATURE - Xaa at position 2 is apartimide or aminosuccinimide.
QXGLAG

SEQ ID NO: 110 - protein, 5 aa, synthetic construct
  REGION 1..5: note = Example 119
  SITE 1: note = MISC_FEATURE - P at position 1 is (2S,4R) trans-4-hydroxy-L-proline.
PGQAV

SEQ ID NO: 111 - protein, 5 aa, synthetic construct
  REGION 1..5: note = Example 120
  SITE 1: note = MISC_FEATURE - P at position 1 is (2S,4R) trans-4-hydroxy-L-proline.
PGQAL

SEQ ID NO: 112 - protein, 5 aa, synthetic construct
  REGION 1..5: note = Example 121
  SITE 1: note = MISC_FEATURE - P at position 1 is (2S,4R) trans-4-hydroxy-L-proline.
PGQLL

SEQ ID NO: 113 - protein, 6 aa, synthetic construct
  REGION 1..6: note = Example 122
  SITE 1: note = MISC_FEATURE - P at position 1 is (2S,4R) trans-4-hydroxy-L-proline.
PGQAGL

SEQ ID NO: 114 - protein, 6 aa, synthetic construct
  REGION 1..6: note = Example 123
  SITE 1: note = MISC_FEATURE - P at position 1 is (2S,4R) trans-4-hydroxy-L-proline.
PGQALL

SEQ ID NO: 115 - protein, 6 aa, synthetic construct
  REGION 1..6: note = Example 124
  SITE 1: note = MISC_FEATURE - P at position 1 is (2S,4R) trans-4-hydroxy-L-proline.
PGQAVL

SEQ ID NO: 116 - protein, 5 aa, synthetic construct
  REGION 1..5: note = Example 125
  SITE 1: note = MISC_FEATURE - P at position 1 is (2S,4R) trans-4-hydroxy-L-proline.
  SITE 4: note = MISC_FEATURE - D at position 4 is D-aspartic acid.
PGQDL